European Patent Specification EP 3 522 699 B1, published December 10, 2025. Title: WHITE RUST RESISTANT CHRYSANTHEMUM PLANTS. Applicant: DÜMMEN GROUP B.V. The sequence listing filed with the application follows.

SEQUENCE LISTING (15 sequences)

SEQ ID NO: 1 - DNA, 192 bp, Chrysanthemum <genus>
  Sequence around 29TgR2
ttaactcaaaaatatgactacaaatcaattttcaggactttttttcgatacttccctctttggtaccggtaccgtattagtggtaccgattttttttgggctcaattcatggtacaggcaccgtaccgtgtattgggagtcggtaccgtttcgatacggtaccggtacggttccgattcgataccggaattc

SEQ ID NO: 2 - DNA, 180 bp, Chrysanthemum <genus>
  Sequence around 24Hs1R1
gaattcctatacgaaggttttgtagatgtgtctccgagcgagtttgatcctaactcacgactagtaatttatgtccataaaaccgataacttgaacattccctcttgttcttgtagatggggatgacttcactgagtctccattcttctggcatcttatcactggaaaaaatcttgttaa

SEQ ID NO: 3 - DNA, 58 bp, Chrysanthemum <genus>
agcaaaacatgcagtgatttatcctcgttaagtgtatggaaaatcgacaccagggtgc

SEQ ID NO: 4 - DNA, 58 bp, Chrysanthemum <genus>
accaaaacaggcagtgatttatcctcgttaagtgtatggaagatcgacaccagagtgc

SEQ ID NO: 5 - DNA, 58 bp, Chrysanthemum <genus>
agcaaaacaggcagtgatttatcctcgttaagtgtatggaagatcgacaccagagtgc

SEQ ID NO: 6 - DNA, 58 bp, Chrysanthemum <genus>
accaaaacaggcagtgatttatcctcgttaagtgtacggaagatcgacagcagggtgc

SEQ ID NO: 7 - DNA, 58 bp, Chrysanthemum <genus>
accaaaacaggcagtgatttatcctcgttaagtgtacggaagatagacagcagggtgc

SEQ ID NO: 8 - DNA, 58 bp, Chrysanthemum <genus>
agcaaaacaggcagtgatttatcctcgttaagtgtatggaagatcgacaccagggtgg

SEQ ID NO: 9 - DNA, 58 bp, Chrysanthemum <genus>
accaaaacaggcagtgatttatcctcgttaagtgtatggaagatcgacaccagggtgg

SEQ ID NO: 10 - DNA, 43 bp, Chrysanthemum <genus>
gaaggtgaccaagttcatgctcaagtcttgtacaaycaaggag

SEQ ID NO: 11 - DNA, 43 bp, Chrysanthemum <genus>
gaaggtcggagtcaacggattcaagtcttgtacaaycaaggac

SEQ ID NO: 12 - DNA, 23 bp, Chrysanthemum <genus>
tacacttaacgaggataaatcac

SEQ ID NO: 13 - DNA, 42 bp, Chrysanthemum <genus>
gaaggtgaccaagttcatgcttacaaccaaggascaaaacat

SEQ ID NO: 14 - DNA, 42 bp, Chrysanthemum <genus>
gaaggtcggagtcaacggatttacaaccaaggascaaaacag

SEQ ID NO: 15 - DNA, 23 bp, Chrysanthemum <genus>
gtcgattttccatacacttaacg